European Patent Specification EP 3 884 022 B1, published June 12, 2024. Title: Detergent Composition. Applicant: Unilever. The sequence listing filed with the application follows.

SEQUENCE LISTING (2 sequences)

SEQ ID NO: 1 - protein, 356 aa, Methanosarcina thermophila
MDDRVSSKQFSGNQVLNGQIPGDEMLKGVNGQIPGDEMLKGVELAIQKSSNFIISNQAGEGYWLDFYILGMGKSSQWVTAYIAYNLSRLPNTDESVQKAIIWLLHTKFPSGGWGYHQNCLPDADSTANTVRLLAYYFKKENLLTQENFALYLHEFARMLSFYQDKNTGGFLTYLPGSNGKYHTMPDSAWCISEPSITAMAGSAFLNAGPELFEQEISSARKFLISRQNPAGYWDSYWWDCRIYGTSLACSFLKQLGETDPVEKAISWLKSIFVPSKGWGNGYEAVPYPFYTALSLSSLLLYEDNVHSREVKESLIWLVENQNEDGSWFSKPILRVPDPQVQEPWESSNREKCEVVT

SEQ ID NO: 2 - protein, 388 aa, Methanosarcina thermophila
MDDRVSSKQFSGNQVLNGQIPGDEMLKGVNGQIPGDEMLKGVELAIQKSSNFIISNQAGEGYWLDFYILGMGKSSQWVTAYIAYNLSRLPNTDESVQKAIIWLLHTKFPSGGWGYHQNCLPDADSTANTVRLLAYYFKKENLLTQENFALYLHEFARMLSFYQDKNTGGFLTYLPGSNGKYHTMPDSAWCISEPSITAMAGSAFLNAGPELFEQEISSARKFLISRQNPAGYWDSYWWDCRIYGTSLACSFLKQLGETDPVEKAISWLKSIFVPSKGWGNGYEAVPYPFYTALSLSSLLLYEDNVHSREVKESLIWLVENQNEDGSWFSKPILRVPDPQVQEPWESSNREKCEVVTDVNLLFTTATVMGVLYDFLNLCGYKYRSASQK